European Patent Application EP 4 461 366 A1, published November 13, 2024. Title: T CELL RECEPTOR, AND PREPARATION METHOD AND USE THEREOF. Applicant: SUZHOU INSTITUTE OF SYSTEMS MEDICINE. The sequence listing filed with the application follows.

SEQUENCE LISTING (48 sequences)

SEQ ID NO: 1 - protein, 109 aa, synthetic construct
IQNPEPAVYQLKDPRSQDSTLCLFTDFDSQINVPKTMESGTFITDKTVLDMKAMDSKSNGAIAWSNQTSFTCQDIFKETNATYPSSDVPCDATLTEKSFETDMNLNFQN

SEQ ID NO: 2 - protein, 22 aa, synthetic construct
LSVMGLRILLLKVAGFNLLMTL

SEQ ID NO: 3 - protein, 5 aa, synthetic construct
RLWSS

SEQ ID NO: 4 - protein, 5 aa, synthetic construct
RLWAA

SEQ ID NO: 5 - protein, 136 aa, synthetic construct
IQNPEPAVYQLKDPRSQDSTLCLFTDFDSQINVPKTMESGTFITDKTVLDMKAMDSKSNGAIAWSNQTSFTCQDIFKETNATYPSSDVPCDATLTEKSFETDMNLNFQNLSVMGLRILLLKVAGFNLLMTLRLWSS

SEQ ID NO: 6 - protein, 136 aa, synthetic construct
IQNPEPAVYQLKDPRSQDSTLCLFTDFDSQINVPKTMESGTFITDKTVLDMKAMDSKSNGAIAWSNQTSFTCQDIFKETNATYPSSDVPCDATLTEKSFETDMNLNFQNLSVMGLRILLLKVAGFNLLMTLRLWAA

SEQ ID NO: 7 - protein, 140 aa, synthetic construct
LRNVTPPKVSLFEPSKAEIANKQKATLVCLARGFFPDHVELSWWVNGKEVHSGVSTDPQAYKESNYSYCLSSRLRVSATFWHNPRNHFRCQVQFHGLSEEDKWPEGSPKPVTQNISAEAWGRADCGITSASYHQGVLSAT

SEQ ID NO: 8 - protein, 22 aa, synthetic construct
ILYEILLGKATLYAVLVSGLVL

SEQ ID NO: 9 - protein, 9 aa, synthetic construct
MAMVKKKNS

SEQ ID NO: 10 - protein, 9 aa, synthetic construct
MAMVRKRNS

SEQ ID NO: 11 - protein, 171 aa, synthetic construct
LRNVTPPKVSLFEPSKAEIANKQKATLVCLARGFFPDHVELSWWVNGKEVHSGVSTDPQAYKESNYSYCLSSRLRVSATFWHNPRNHFRCQVQFHGLSEEDKWPEGSPKPVTQNISAEAWGRADCGITSASYHQGVLSATILYEILLGKATLYAVLVSGLVLMAMVKKKNS

SEQ ID NO: 12 - protein, 171 aa, synthetic construct
LRNVTPPKVSLFEPSKAEIANKQKATLVCLARGFFPDHVELSWWVNGKEVHSGVSTDPQAYKESNYSYCLSSRLRVSATFWHNPRNHFRCQVQFHGLSEEDKWPEGSPKPVTQNISAEAWGRADCGITSASYHQGVLSATILYEILLGKATLYAVLVSGLVLMAMVRKRNS

SEQ ID NO: 13 - protein, 112 aa, synthetic construct
QQKEVEQNSGPLSVPEGAIASLNCTYSDRGSQSFFWYRQYSGKSPELIMFIYSNGDKEDGRFTAQLNKASQYVSLLIRDSQPSDSATYLCAVNFGGGKLIFGQGTELSVKPN

SEQ ID NO: 14 - protein, 6 aa, synthetic construct
DRGSQS

SEQ ID NO: 15 - protein, 6 aa, synthetic construct
IYSNGD

SEQ ID NO: 16 - protein, 10 aa, synthetic construct
AVNFGGGKLI

SEQ ID NO: 17 - protein, 112 aa, synthetic construct
GITQAPTSQILAAGRRMTLRCTQDMRHNAMYWYRQDLGLGLRLIHYSNTAGTTGKGEVPDGYSVSRANTDDFPLTLASAVPSQTSVYFCASSLSFGTEAFFGQGTRLTVVED

SEQ ID NO: 18 - protein, 5 aa, synthetic construct
MRHNA

SEQ ID NO: 19 - protein, 6 aa, synthetic construct
SNTAGT

SEQ ID NO: 20 - protein, 11 aa, synthetic construct
ASSLSFGTEAF

SEQ ID NO: 21 - protein, 115 aa, synthetic construct
KQEVTQIPAALSVPEGENLVLNCSFTDSAIYNLQWFRQDPGKGLTSLLLIQSSQREQTSGRLNASLDKSSGRSTLYIAASQPGDSATYLCAVRPTSGGSYIPTFGRGTSLIVHPY

SEQ ID NO: 22 - protein, 6 aa, synthetic construct
DSAIYN

SEQ ID NO: 23 - protein, 5 aa, synthetic construct
IQSSQ

SEQ ID NO: 24 - protein, 10 aa, synthetic construct
PTSGGSYIPT

SEQ ID NO: 25 - protein, 113 aa, synthetic construct
GVTQTPKFQVLKTGQSMTLQCAQDMNHEYMSWYRQDPGMGLRLIHYSVGAGITDQGEVPNGYNVSRSTTEDFPLRLLSAAPSQTSVYFCASSYVGNTGELFFGEGSRLTVLED

SEQ ID NO: 26 - protein, 5 aa, synthetic construct
MNHEY

SEQ ID NO: 27 - protein, 4 aa, synthetic construct
GAGI

SEQ ID NO: 28 - protein, 4 aa, synthetic construct
YVGN

SEQ ID NO: 29 - protein, 26 aa, synthetic construct
MATGSRTSLLLAFGLLCLPWLQEASA

SEQ ID NO: 30 - protein, 26 aa, synthetic construct
MATGSRTSLLLAFGLLCLPCLQEGSA

SEQ ID NO: 31 - DNA, 408 bp, synthetic construct
  source 1..408: mol_type = other DNA
atccagaaccccgagcccgccgtgtaccagctgaaggaccccagaagccaggacagcaccctgtgcctgttcaccgacttcgacagccagatcaacgtgcccaagaccatggagagcggcaccttcatcaccgacaagaccgtgctggacatgaaggccatggacagcaagagcaacggcgccatcgcctggtccaaccagaccagcttcacatgccaggacatcttcaaggagaccaacgccacctaccccagcagcgacgtgccctgcgacgccaccctgaccgagaagagcttcgagaccgacatgaacctgaacttccagaacctgagcgtgatgggcctgagaatcctgctgctgaaggtggccggcttcaacctgctgatgaccctgaggctgtggagcagc

SEQ ID NO: 32 - DNA, 513 bp, synthetic construct
  source 1..513: mol_type = other DNA
ctgaggaacgtgaccccccccaaggtgtccctgttcgagcccagcaaggccgagatcgccaacaagcagaaggccaccctggtgtgcctggccaggggcttcttccccgaccacgtggagctgtcttggtgggtgaacggcaaggaggtgcacagcggcgtgagcaccgacccccaggcctacaaggagagcaactacagctactgcctgagcagcaggctgagagtgagcgccaccttctggcacaaccccaggaaccacttccgctgtcaggtgcagttccacggcctgagcgaggaggacaagtggcccgagggcagccccaagcccgtgacccagaacatcagcgccgaggcctggggcagagccgactgcggcatcaccagcgccagctaccaccagggcgtgctgtccgccaccatcctgtacgagatcctgctgggcaaggccacactgtacgccgtgctggtgtccggcctggtgctgatggccatggtgaagaagaagaacagc

SEQ ID NO: 33 - DNA, 408 bp, synthetic construct
  source 1..408: mol_type = other DNA
atccagaaccccgagcccgccgtgtaccagctgaaggaccccagaagccaggacagcaccctgtgcctgttcaccgacttcgacagccagatcaacgtgcccaagaccatggagagcggcaccttcatcaccgacaagaccgtgctggacatgaaggccatggacagcaagagcaacggcgccatcgcctggtccaaccagaccagcttcacatgccaggacatcttcaaggagaccaacgccacctaccccagcagcgacgtgccctgcgacgccaccctgaccgagaagagcttcgagaccgacatgaacctgaacttccagaacctgagcgtgatgggcctgagaatcctgctgctgaaggtggccggcttcaacctgctgatgaccctgaggctgtgggccgcc

SEQ ID NO: 34 - DNA, 513 bp, synthetic construct
  source 1..513: mol_type = other DNA
ctgaggaacgtgaccccccccaaggtgtccctgttcgagcccagcaaggccgagatcgccaacaagcagaaggccaccctggtgtgcctggccaggggcttcttccccgaccacgtggagctgtcttggtgggtgaacggcaaggaggtgcacagcggcgtgagcaccgacccccaggcctacaaggagagcaactacagctactgcctgagcagcaggctgagagtgagcgccaccttctggcacaaccccaggaaccacttccgctgtcaggtgcagttccacggcctgagcgaggaggacaagtggcccgagggcagccccaagcccgtgacccagaacatcagcgccgaggcctggggcagagccgactgcggcatcaccagcgccagctaccaccagggcgtgctgtccgccaccatcctgtacgagatcctgctgggcaaggccacactgtacgccgtgctggtgtccggcctggtgctgatggccatggtgaggaagaggaacagc

SEQ ID NO: 35 - DNA, 336 bp, synthetic construct
  source 1..336: mol_type = other DNA
caacagaaggaggtggagcagaattctggacccctcagtgttccagagggagccattgcctctctcaactgcacttacagtgaccgaggttcccagtccttcttctggtacagacaatattctgggaaaagccctgagttgataatgttcatatactccaatggtgacaaagaagatggaaggtttacagcacagctcaataaagccagccagtatgtttctctgctcatcagagactcccagcccagtgattcagccacctacctctgtgccgtgaacttcggaggaggaaagcttatcttcggacagggaacggagttatctgtgaaacccaat

SEQ ID NO: 36 - DNA, 336 bp, synthetic construct
  source 1..336: mol_type = other DNA
gggatcacccaggcaccaacatctcagatcctggcagcaggacggcgcatgacactgagatgtacccaggatatgagacataatgccatgtactggtatagacaagatctaggactggggctaaggctcatccattattcaaatactgcaggtaccactggcaaaggagaagtccctgatggttatagtgtctccagagcaaacacagatgatttccccctcacgttggcgtctgctgtaccctctcagacatctgtgtacttctgtgccagcagcctaagtttcggcactgaagctttctttggacaaggcaccagactcacagttgtagaggac

SEQ ID NO: 37 - DNA, 345 bp, synthetic construct
  source 1..345: mol_type = other DNA
aaacaggaggtgacgcagattcctgcagctctgagtgtcccagaaggagaaaacttggttctcaactgcagtttcactgatagcgctatttacaacctccagtggtttaggcaggaccctgggaaaggtctcacatctctgttgcttattcagtcaagtcagagagagcaaacaagtggaagacttaatgcctcgctggataaatcatcaggacgtagtactttatacattgcagcttctcagcctggtgactcagccacctacctctgtgctgtgaggcccacatcaggaggaagctacatacctacatttggaagaggaaccagccttattgttcatccgtat

SEQ ID NO: 38 - DNA, 339 bp, synthetic construct
  source 1..339: mol_type = other DNA
ggtgtcactcagaccccaaaattccaggtcctgaagacaggacagagcatgacactgcagtgtgcccaggatatgaaccatgaatacatgtcctggtatcgacaagacccaggcatggggctgaggctgattcattactcagttggtgctggtatcactgaccaaggagaagtccccaatggctacaatgtctccagatcaaccacagaggatttcccgctcaggctgctgtcggctgctccctcccagacatctgtgtacttctgtgccagcagttacgtcgggaacaccggggagctgttttttggagaaggctctaggctgaccgtactggaggac

SEQ ID NO: 39 - DNA, 1848 bp, synthetic construct
  source 1..1848: mol_type = other DNA
atggcgacgggttcaagaacttccctacttcttgcatttggcctgctttgtttgccgtggttacaggaagcctcagcacaacagaaggaggtggagcagaattctggacccctcagtgttccagagggagccattgcctctctcaactgcacttacagtgaccgaggttcccagtccttcttctggtacagacaatattctgggaaaagccctgagttgataatgttcatatactccaatggtgacaaagaagatggaaggtttacagcacagctcaataaagccagccagtatgtttctctgctcatcagagactcccagcccagtgattcagccacctacctctgtgccgtgaacttcggaggaggaaagcttatcttcggacagggaacggagttatctgtgaaacccaatatccagaaccccgagcccgccgtgtaccagctgaaggaccccagaagccaggacagcaccctgtgcctgttcaccgacttcgacagccagatcaacgtgcccaagaccatggagagcggcaccttcatcaccgacaagaccgtgctggacatgaaggccatggacagcaagagcaacggcgccatcgcctggtccaaccagaccagcttcacatgccaggacatcttcaaggagaccaacgccacctaccccagcagcgacgtgccctgcgacgccaccctgaccgagaagagcttcgagaccgacatgaacctgaacttccagaacctgagcgtgatgggcctgagaatcctgctgctgaaggtggccggcttcaacctgctgatgaccctgaggctgtggagcagcagggcaaaacgttcgggttcgggtgcgccagtaaagcagacattaaactttgatttgctgaaacttgcaggtgatgtagagtcaaatccaggtccaatggcaacagggagccgaacctctctgctccttgctttcgggctcctttgcctaccgtgcctgcaggagggctcggcagggatcacccaggcaccaacatctcagatcctggcagcaggacggcgcatgacactgagatgtacccaggatatgagacataatgccatgtactggtatagacaagatctaggactggggctaaggctcatccattattcaaatactgcaggtaccactggcaaaggagaagtccctgatggttatagtgtctccagagcaaacacagatgatttccccctcacgttggcgtctgctgtaccctctcagacatctgtgtacttctgtgccagcagcctaagtttcggcactgaagctttctttggacaaggcaccagactcacagttgtagaggacctgaggaacgtgaccccccccaaggtgtccctgttcgagcccagcaaggccgagatcgccaacaagcagaaggccaccctggtgtgcctggccaggggcttcttccccgaccacgtggagctgtcttggtgggtgaacggcaaggaggtgcacagcggcgtgagcaccgacccccaggcctacaaggagagcaactacagctactgcctgagcagcaggctgagagtgagcgccaccttctggcacaaccccaggaaccacttccgctgtcaggtgcagttccacggcctgagcgaggaggacaagtggcccgagggcagccccaagcccgtgacccagaacatcagcgccgaggcctggggcagagccgactgcggcatcaccagcgccagctaccaccagggcgtgctgtccgccaccatcctgtacgagatcctgctgggcaaggccacactgtacgccgtgctggtgtccggcctggtgctgatggccatggtgaagaagaagaacagctaa

SEQ ID NO: 40 - DNA, 1848 bp, synthetic construct
  source 1..1848: mol_type = other DNA
atggcgacgggttcaagaacttccctacttcttgcatttggcctgctttgtttgccgtggttacaggaagcctcagcacaacagaaggaggtggagcagaattctggacccctcagtgttccagagggagccattgcctctctcaactgcacttacagtgaccgaggttcccagtccttcttctggtacagacaatattctgggaaaagccctgagttgataatgttcatatactccaatggtgacaaagaagatggaaggtttacagcacagctcaataaagccagccagtatgtttctctgctcatcagagactcccagcccagtgattcagccacctacctctgtgccgtgaacttcggaggaggaaagcttatcttcggacagggaacggagttatctgtgaaacccaatatccagaaccccgagcccgccgtgtaccagctgaaggaccccagaagccaggacagcaccctgtgcctgttcaccgacttcgacagccagatcaacgtgcccaagaccatggagagcggcaccttcatcaccgacaagaccgtgctggacatgaaggccatggacagcaagagcaacggcgccatcgcctggtccaaccagaccagcttcacatgccaggacatcttcaaggagaccaacgccacctaccccagcagcgacgtgccctgcgacgccaccctgaccgagaagagcttcgagaccgacatgaacctgaacttccagaacctgagcgtgatgggcctgagaatcctgctgctgaaggtggccggcttcaacctgctgatgaccctgaggctgtgggccgccagggcaaaacgttcgggttcgggtgcgccagtaaagcagacattaaactttgatttgctgaaacttgcaggtgatgtagagtcaaatccaggtccaatggcaacagggagccgaacctctctgctccttgctttcgggctcctttgcctaccgtgcctgcaggagggctcggcagggatcacccaggcaccaacatctcagatcctggcagcaggacggcgcatgacactgagatgtacccaggatatgagacataatgccatgtactggtatagacaagatctaggactggggctaaggctcatccattattcaaatactgcaggtaccactggcaaaggagaagtccctgatggttatagtgtctccagagcaaacacagatgatttccccctcacgttggcgtctgctgtaccctctcagacatctgtgtacttctgtgccagcagcctaagtttcggcactgaagctttctttggacaaggcaccagactcacagttgtagaggacctgaggaacgtgaccccccccaaggtgtccctgttcgagcccagcaaggccgagatcgccaacaagcagaaggccaccctggtgtgcctggccaggggcttcttccccgaccacgtggagctgtcttggtgggtgaacggcaaggaggtgcacagcggcgtgagcaccgacccccaggcctacaaggagagcaactacagctactgcctgagcagcaggctgagagtgagcgccaccttctggcacaaccccaggaaccacttccgctgtcaggtgcagttccacggcctgagcgaggaggacaagtggcccgagggcagccccaagcccgtgacccagaacatcagcgccgaggcctggggcagagccgactgcggcatcaccagcgccagctaccaccagggcgtgctgtccgccaccatcctgtacgagatcctgctgggcaaggccacactgtacgccgtgctggtgtccggcctggtgctgatggccatggtgaagaagaagaacagctaa

SEQ ID NO: 41 - DNA, 1848 bp, synthetic construct; identical to SEQ ID NO: 40
  source 1..1848: mol_type = other DNA

SEQ ID NO: 42 - DNA, 1848 bp, synthetic construct
  source 1..1848: mol_type = other DNA
atggcgacgggttcaagaacttccctacttcttgcatttggcctgctttgtttgccgtggttacaggaagcctcagcacaacagaaggaggtggagcagaattctggacccctcagtgttccagagggagccattgcctctctcaactgcacttacagtgaccgaggttcccagtccttcttctggtacagacaatattctgggaaaagccctgagttgataatgttcatatactccaatggtgacaaagaagatggaaggtttacagcacagctcaataaagccagccagtatgtttctctgctcatcagagactcccagcccagtgattcagccacctacctctgtgccgtgaacttcggaggaggaaagcttatcttcggacagggaacggagttatctgtgaaacccaatatccagaaccccgagcccgccgtgtaccagctgaaggaccccagaagccaggacagcaccctgtgcctgttcaccgacttcgacagccagatcaacgtgcccaagaccatggagagcggcaccttcatcaccgacaagaccgtgctggacatgaaggccatggacagcaagagcaacggcgccatcgcctggtccaaccagaccagcttcacatgccaggacatcttcaaggagaccaacgccacctaccccagcagcgacgtgccctgcgacgccaccctgaccgagaagagcttcgagaccgacatgaacctgaacttccagaacctgagcgtgatgggcctgagaatcctgctgctgaaggtggccggcttcaacctgctgatgaccctgaggctgtgggccgccagggcaaaacgttcgggttcgggtgcgccagtaaagcagacattaaactttgatttgctgaaacttgcaggtgatgtagagtcaaatccaggtccaatggcaacagggagccgaacctctctgctccttgctttcgggctcctttgcctaccgtgcctgcaggagggctcggcagggatcacccaggcaccaacatctcagatcctggcagcaggacggcgcatgacactgagatgtacccaggatatgagacataatgccatgtactggtatagacaagatctaggactggggctaaggctcatccattattcaaatactgcaggtaccactggcaaaggagaagtccctgatggttatagtgtctccagagcaaacacagatgatttccccctcacgttggcgtctgctgtaccctctcagacatctgtgtacttctgtgccagcagcctaagtttcggcactgaagctttctttggacaaggcaccagactcacagttgtagaggacctgaggaacgtgaccccccccaaggtgtccctgttcgagcccagcaaggccgagatcgccaacaagcagaaggccaccctggtgtgcctggccaggggcttcttccccgaccacgtggagctgtcttggtgggtgaacggcaaggaggtgcacagcggcgtgagcaccgacccccaggcctacaaggagagcaactacagctactgcctgagcagcaggctgagagtgagcgccaccttctggcacaaccccaggaaccacttccgctgtcaggtgcagttccacggcctgagcgaggaggacaagtggcccgagggcagccccaagcccgtgacccagaacatcagcgccgaggcctggggcagagccgactgcggcatcaccagcgccagctaccaccagggcgtgctgtccgccaccatcctgtacgagatcctgctgggcaaggccacactgtacgccgtgctggtgtccggcctggtgctgatggccatggtgaggaagaggaacagctaa

SEQ ID NO: 43 - DNA, 1860 bp, synthetic construct
  source 1..1860: mol_type = other DNA
atggcgacgggttcaagaacttccctacttcttgcatttggcctgctttgtttgccgtggttacaggaagcctcagcaaaacaggaggtgacgcagattcctgcagctctgagtgtcccagaaggagaaaacttggttctcaactgcagtttcactgatagcgctatttacaacctccagtggtttaggcaggaccctgggaaaggtctcacatctctgttgcttattcagtcaagtcagagagagcaaacaagtggaagacttaatgcctcgctggataaatcatcaggacgtagtactttatacattgcagcttctcagcctggtgactcagccacctacctctgtgctgtgaggcccacatcaggaggaagctacatacctacatttggaagaggaaccagccttattgttcatccgtatatccagaaccccgagcccgccgtgtaccagctgaaggaccccagaagccaggacagcaccctgtgcctgttcaccgacttcgacagccagatcaacgtgcccaagaccatggagagcggcaccttcatcaccgacaagaccgtgctggacatgaaggccatggacagcaagagcaacggcgccatcgcctggtccaaccagaccagcttcacatgccaggacatcttcaaggagaccaacgccacctaccccagcagcgacgtgccctgcgacgccaccctgaccgagaagagcttcgagaccgacatgaacctgaacttccagaacctgagcgtgatgggcctgagaatcctgctgctgaaggtggccggcttcaacctgctgatgaccctgaggctgtggagcagcagggcaaaacgttcgggttcgggtgcgccagtaaagcagacattaaactttgatttgctgaaacttgcaggtgatgtagagtcaaatccaggtccaatggcaacagggagccgaacctctctgctccttgctttcgggctcctttgcctaccgtgcctgcaggagggctcggcaggtgtcactcagaccccaaaattccaggtcctgaagacaggacagagcatgacactgcagtgtgcccaggatatgaaccatgaatacatgtcctggtatcgacaagacccaggcatggggctgaggctgattcattactcagttggtgctggtatcactgaccaaggagaagtccccaatggctacaatgtctccagatcaaccacagaggatttcccgctcaggctgctgtcggctgctccctcccagacatctgtgtacttctgtgccagcagttacgtcgggaacaccggggagctgttttttggagaaggctctaggctgaccgtactggaggacctgaggaacgtgaccccccccaaggtgtccctgttcgagcccagcaaggccgagatcgccaacaagcagaaggccaccctggtgtgcctggccaggggcttcttccccgaccacgtggagctgtcttggtgggtgaacggcaaggaggtgcacagcggcgtgagcaccgacccccaggcctacaaggagagcaactacagctactgcctgagcagcaggctgagagtgagcgccaccttctggcacaaccccaggaaccacttccgctgtcaggtgcagttccacggcctgagcgaggaggacaagtggcccgagggcagccccaagcccgtgacccagaacatcagcgccgaggcctggggcagagccgactgcggcatcaccagcgccagctaccaccagggcgtgctgtccgccaccatcctgtacgagatcctgctgggcaaggccacactgtacgccgtgctggtgtccggcctggtgctgatggccatggtgaagaagaagaacagctaa

SEQ ID NO: 44 - DNA, 1860 bp, synthetic construct
  source 1..1860: mol_type = other DNA
atggcgacgggttcaagaacttccctacttcttgcatttggcctgctttgtttgccgtggttacaggaagcctcagcaaaacaggaggtgacgcagattcctgcagctctgagtgtcccagaaggagaaaacttggttctcaactgcagtttcactgatagcgctatttacaacctccagtggtttaggcaggaccctgggaaaggtctcacatctctgttgcttattcagtcaagtcagagagagcaaacaagtggaagacttaatgcctcgctggataaatcatcaggacgtagtactttatacattgcagcttctcagcctggtgactcagccacctacctctgtgctgtgaggcccacatcaggaggaagctacatacctacatttggaagaggaaccagccttattgttcatccgtatatccagaaccccgagcccgccgtgtaccagctgaaggaccccagaagccaggacagcaccctgtgcctgttcaccgacttcgacagccagatcaacgtgcccaagaccatggagagcggcaccttcatcaccgacaagaccgtgctggacatgaaggccatggacagcaagagcaacggcgccatcgcctggtccaaccagaccagcttcacatgccaggacatcttcaaggagaccaacgccacctaccccagcagcgacgtgccctgcgacgccaccctgaccgagaagagcttcgagaccgacatgaacctgaacttccagaacctgagcgtgatgggcctgagaatcctgctgctgaaggtggccggcttcaacctgctgatgaccctgaggctgtgggccgccagggcaaaacgttcgggttcgggtgcgccagtaaagcagacattaaactttgatttgctgaaacttgcaggtgatgtagagtcaaatccaggtccaatggcaacagggagccgaacctctctgctccttgctttcgggctcctttgcctaccgtgcctgcaggagggctcggcaggtgtcactcagaccccaaaattccaggtcctgaagacaggacagagcatgacactgcagtgtgcccaggatatgaaccatgaatacatgtcctggtatcgacaagacccaggcatggggctgaggctgattcattactcagttggtgctggtatcactgaccaaggagaagtccccaatggctacaatgtctccagatcaaccacagaggatttcccgctcaggctgctgtcggctgctccctcccagacatctgtgtacttctgtgccagcagttacgtcgggaacaccggggagctgttttttggagaaggctctaggctgaccgtactggaggacctgaggaacgtgaccccccccaaggtgtccctgttcgagcccagcaaggccgagatcgccaacaagcagaaggccaccctggtgtgcctggccaggggcttcttccccgaccacgtggagctgtcttggtgggtgaacggcaaggaggtgcacagcggcgtgagcaccgacccccaggcctacaaggagagcaactacagctactgcctgagcagcaggctgagagtgagcgccaccttctggcacaaccccaggaaccacttccgctgtcaggtgcagttccacggcctgagcgaggaggacaagtggcccgagggcagccccaagcccgtgacccagaacatcagcgccgaggcctggggcagagccgactgcggcatcaccagcgccagctaccaccagggcgtgctgtccgccaccatcctgtacgagatcctgctgggcaaggccacactgtacgccgtgctggtgtccggcctggtgctgatggccatggtgaagaagaagaacagctaa

SEQ ID NO: 45 - DNA, 1860 bp, synthetic construct
  source 1..1860: mol_type = other DNA
atggcgacgggttcaagaacttccctacttcttgcatttggcctgctttgtttgccgtggttacaggaagcctcagcaaaacaggaggtgacgcagattcctgcagctctgagtgtcccagaaggagaaaacttggttctcaactgcagtttcactgatagcgctatttacaacctccagtggtttaggcaggaccctgggaaaggtctcacatctctgttgcttattcagtcaagtcagagagagcaaacaagtggaagacttaatgcctcgctggataaatcatcaggacgtagtactttatacattgcagcttctcagcctggtgactcagccacctacctctgtgctgtgaggcccacatcaggaggaagctacatacctacatttggaagaggaaccagccttattgttcatccgtatatccagaaccccgagcccgccgtgtaccagctgaaggaccccagaagccaggacagcaccctgtgcctgttcaccgacttcgacagccagatcaacgtgcccaagaccatggagagcggcaccttcatcaccgacaagaccgtgctggacatgaaggccatggacagcaagagcaacggcgccatcgcctggtccaaccagaccagcttcacatgccaggacatcttcaaggagaccaacgccacctaccccagcagcgacgtgccctgcgacgccaccctgaccgagaagagcttcgagaccgacatgaacctgaacttccagaacctgagcgtgatgggcctgagaatcctgctgctgaaggtggccggcttcaacctgctgatgaccctgaggctgtggagcagcagggcaaaacgttcgggttcgggtgcgccagtaaagcagacattaaactttgatttgctgaaacttgcaggtgatgtagagtcaaatccaggtccaatggcaacagggagccgaacctctctgctccttgctttcgggctcctttgcctaccgtgcctgcaggagggctcggcaggtgtcactcagaccccaaaattccaggtcctgaagacaggacagagcatgacactgcagtgtgcccaggatatgaaccatgaatacatgtcctggtatcgacaagacccaggcatggggctgaggctgattcattactcagttggtgctggtatcactgaccaaggagaagtccccaatggctacaatgtctccagatcaaccacagaggatttcccgctcaggctgctgtcggctgctccctcccagacatctgtgtacttctgtgccagcagttacgtcgggaacaccggggagctgttttttggagaaggctctaggctgaccgtactggaggacctgaggaacgtgaccccccccaaggtgtccctgttcgagcccagcaaggccgagatcgccaacaagcagaaggccaccctggtgtgcctggccaggggcttcttccccgaccacgtggagctgtcttggtgggtgaacggcaaggaggtgcacagcggcgtgagcaccgacccccaggcctacaaggagagcaactacagctactgcctgagcagcaggctgagagtgagcgccaccttctggcacaaccccaggaaccacttccgctgtcaggtgcagttccacggcctgagcgaggaggacaagtggcccgagggcagccccaagcccgtgacccagaacatcagcgccgaggcctggggcagagccgactgcggcatcaccagcgccagctaccaccagggcgtgctgtccgccaccatcctgtacgagatcctgctgggcaaggccacactgtacgccgtgctggtgtccggcctggtgctgatggccatggtgaggaagaggaacagctaa

SEQ ID NO: 46 - DNA, 1860 bp, synthetic construct
  source 1..1860: mol_type = other DNA
atggcgacgggttcaagaacttccctacttcttgcatttggcctgctttgtttgccgtggttacaggaagcctcagcaaaacaggaggtgacgcagattcctgcagctctgagtgtcccagaaggagaaaacttggttctcaactgcagtttcactgatagcgctatttacaacctccagtggtttaggcaggaccctgggaaaggtctcacatctctgttgcttattcagtcaagtcagagagagcaaacaagtggaagacttaatgcctcgctggataaatcatcaggacgtagtactttatacattgcagcttctcagcctggtgactcagccacctacctctgtgctgtgaggcccacatcaggaggaagctacatacctacatttggaagaggaaccagccttattgttcatccgtatatccagaaccccgagcccgccgtgtaccagctgaaggaccccagaagccaggacagcaccctgtgcctgttcaccgacttcgacagccagatcaacgtgcccaagaccatggagagcggcaccttcatcaccgacaagaccgtgctggacatgaaggccatggacagcaagagcaacggcgccatcgcctggtccaaccagaccagcttcacatgccaggacatcttcaaggagaccaacgccacctaccccagcagcgacgtgccctgcgacgccaccctgaccgagaagagcttcgagaccgacatgaacctgaacttccagaacctgagcgtgatgggcctgagaatcctgctgctgaaggtggccggcttcaacctgctgatgaccctgaggctgtgggccgccagggcaaaacgttcgggttcgggtgcgccagtaaagcagacattaaactttgatttgctgaaacttgcaggtgatgtagagtcaaatccaggtccaatggcaacagggagccgaacctctctgctccttgctttcgggctcctttgcctaccgtgcctgcaggagggctcggcaggtgtcactcagaccccaaaattccaggtcctgaagacaggacagagcatgacactgcagtgtgcccaggatatgaaccatgaatacatgtcctggtatcgacaagacccaggcatggggctgaggctgattcattactcagttggtgctggtatcactgaccaaggagaagtccccaatggctacaatgtctccagatcaaccacagaggatttcccgctcaggctgctgtcggctgctccctcccagacatctgtgtacttctgtgccagcagttacgtcgggaacaccggggagctgttttttggagaaggctctaggctgaccgtactggaggacctgaggaacgtgaccccccccaaggtgtccctgttcgagcccagcaaggccgagatcgccaacaagcagaaggccaccctggtgtgcctggccaggggcttcttccccgaccacgtggagctgtcttggtgggtgaacggcaaggaggtgcacagcggcgtgagcaccgacccccaggcctacaaggagagcaactacagctactgcctgagcagcaggctgagagtgagcgccaccttctggcacaaccccaggaaccacttccgctgtcaggtgcagttccacggcctgagcgaggaggacaagtggcccgagggcagccccaagcccgtgacccagaacatcagcgccgaggcctggggcagagccgactgcggcatcaccagcgccagctaccaccagggcgtgctgtccgccaccatcctgtacgagatcctgctgggcaaggccacactgtacgccgtgctggtgtccggcctggtgctgatggccatggtgaggaagaggaacagctaa

SEQ ID NO: 47 - protein, 11 aa, synthetic construct
MAMVKRKDSRG

SEQ ID NO: 48 - protein, 9 aa, synthetic construct
MAMVKRKDF